European Patent Specification EP 3 256 102 B1, published August 9, 2023. Title: PEPTIDIC COMPOUNDS, COMPOSITIONS COMPRISING THEM AND USES IN PARTICULAR COSMETIC OF SAID COMPOUNDS. Applicant: SEDERMA. The sequence listing filed with the application follows.

SEQUENCE LISTING (20 sequences)

SEQ ID NO: 1 - protein, 5 aa, artificial sequence
  synthetic peptide
  MOD_RES (1)..(1): amidation by a Palmitoyl chain
KTTKS

SEQ ID NO: 2 - protein, 4 aa, artificial sequence
  synthetic peptide
  MOD_RES (1)..(1): amidation by a Palmitoyl chain
GQPR

SEQ ID NO: 3 - protein, 4 aa, artificial sequence
  synthetic peptide
KTFK

SEQ ID NO: 4 - protein, 4 aa, artificial sequence
  synthetic peptide
KGHK

SEQ ID NO: 5 - protein, 6 aa, artificial sequence
  synthetic peptide
GKTTKS

SEQ ID NO: 6 - protein, 4 aa, artificial sequence
  synthetic peptide
RSRK

SEQ ID NO: 7 - protein, 4 aa, artificial sequence
  synthetic peptide
GQPR

SEQ ID NO: 8 - protein, 5 aa, artificial sequence
  synthetic peptide
KTTKS

SEQ ID NO: 9 - protein, 6 aa, artificial sequence
  synthetic peptide
VGVAPG

SEQ ID NO: 10 - protein, 4 aa, artificial sequence
  synthetic peptide
  MOD_RES (1)..(1): amidation by an elaidoyl chain on the N terminal end
KTFK

SEQ ID NO: 11 - protein, 5 aa, artificial sequence
  synthetic peptide
  MOD_RES (1)..(1): Amidation by a Palmitoyl chain
YGGFL

SEQ ID NO: 12 - protein, 5 aa, artificial sequence
  synthetic peptide
  MOD_RES (1)..(1): Amidation by a palmitoyl chain
YGGFP

SEQ ID NO: 13 - protein, 6 aa, artificial sequence
  synthetic peptide
HLDIIW

SEQ ID NO: 14 - protein, 6 aa, artificial sequence
  Synthetic peptide
  MISC_FEATURE (6)..(6): Xaa is aTryptoline-3-carboxylic acid residu (Tpi)
HLDIIX

SEQ ID NO: 15 - protein, 6 aa, artificial sequence
  Synthetic peptide
HLDIIF

SEQ ID NO: 16 - protein, 6 aa, artificial sequence
  synthetic peptide
  MOD_RES (1)..(1): Acetylation
  MOD_RES (6)..(6): NH2
EEMQRR

SEQ ID NO: 17 - protein, 5 aa, artificial sequence
  synthetic peptide
YAGFL

SEQ ID NO: 18 - protein, 4 aa, artificial sequence
  synthetic peptide
  MOD_RES (1)..(1): Acetylation
AHSH

SEQ ID NO: 19 - protein, 6 aa, artificial sequence
  synthetic peptide
SIKVAV

SEQ ID NO: 20 - protein, 6 aa, artificial sequence
  synthetic peptide
GPQGPQ